European Patent Application EP 4 295 911 A2, published December 27, 2023. Title: HUMANIZED ANTI-COMPLEMENT FACTOR C1Q ANTIBODIES AND USES THEREOF. Applicant: ANNEXON, INC. The sequence listing filed with the application follows.

SEQUENCE LISTING (46 sequences)

SEQ ID NO: 1 - protein, 121 aa, synthetic construct [sequence omitted]

SEQ ID NO: 2 - protein, 121 aa, synthetic construct [sequence omitted]

SEQ ID NO: 3 - protein, 121 aa, synthetic construct
QVQLVQSGAELKKPGASVKVSCKSSGYHFTSYWMHWVKQAPGQGLEWIGVIHPNSGSINYNEKFESRVTITVDKSTSTAYMELSSLRSEDTAVYYCAGERDSTEVLPMDYWGQGTTVTVSS

SEQ ID NO: 4 - protein, 121 aa, synthetic construct [sequence omitted]

SEQ ID NO: 5 - protein, 107 aa, synthetic construct [sequence omitted]

SEQ ID NO: 6 - protein, 107 aa, synthetic construct [sequence omitted]

SEQ ID NO: 7 - protein, 107 aa, synthetic construct
DVQITQSPSSLSASLGERATINCRASKSINKYLAWYQQKPGKAPKLLIYSGSTLQSGIPARFSGSGSGTDFTLTISSLEPEDFAMYYCQQHNEYPLTFGQGTKLEIK

SEQ ID NO: 8 - protein, 107 aa, synthetic construct [sequence omitted]

SEQ ID NO: 9 - protein, 245 aa, Homo sapiens
MEGPRGWLVLCVLAISLASMVTEDLCRAPDGKKGEAGRPGRRGRPGLKGEQGEPGAPGIRTGIQGLKGDQGEPGPSGNPGKVGYPGPSGPLGARGIPGIKGTKGSPGNIKDQPRPAFSAIRRNPPMGGNVVIFDTVITNQEEPYQNHSGRFVCTVPGYYYFTFQVLSQWEICLSIVSSSRGQVRRSLGFCDTTNKGLFQVVSGGMVLQLQQGDQVWVEKDPKKGHIYQGSEADSVFSGFLIFPSA

SEQ ID NO: 10 - protein, 253 aa, Homo sapiens
MMMKIPWGSIPVLMLLLLLGLIDISQAQLSCTGPPAIPGIPGIPGTPGPDGQPGTPGIKGEKGLPGLAGDHGEFGEKGDPGIPGNPGKVGPKGPMGPKGGPGAPGAPGPKGESGDYKATQKIAFSATRTINVPLRRDQTIRFDHVITNMNNNYEPRSGKFTCKVPGLYYFTYHASSRGNLCVNLMRGRERAQKVVTFCDYAYNTFQVTTGGMVLKLEQGENVFLQATDKNSLLGMEGANSIFSGFLLFPDMEA

SEQ ID NO: 11 - protein, 245 aa, Homo sapiens
MDVGPSSLPHLGLKLLLLLLLLPLRGQANTGCYGIPGMPGLPGAPGKDGYDGLPGPKGEPGIPAIPGIRGPKGQKGEPGLPGHPGKNGPMGPPGMPGVPGPMGIPGEPGEEGRYKQKFQSVFTVTRQTHQPPAPNSLIRFNAVLTNPQGDYDTSTGKFTCKVPGLYYFVYHASHTANLCVLLYRSGVKVVTFCGHTSKTNQVNSGGVLLRLQVGEEVWLAVNDYYDMVGIQGSDSVFSGFLLFPD

SEQ ID NO: 12 - protein, 31 aa, Homo sapiens
GLFQVVSGGMVLQLQQGDQVWVEKDPKKGHI

SEQ ID NO: 13 - protein, 26 aa, Homo sapiens
GLFQVVSGGMVLQLQQGDQVWVEKDP

SEQ ID NO: 14 - protein, 20 aa, Homo sapiens
SGGMVLQLQQGDQVWVEKDP

SEQ ID NO: 15 - protein, 18 aa, Homo sapiens
SGGMVLQLQQGDQVWVEK

SEQ ID NO: 16 - protein, 23 aa, Homo sapiens
WLAVNDYYDMVGIQGSDSVFSGF

SEQ ID NO: 17 - protein, 16 aa, Homo sapiens
YDMVGIQGSDSVFSGF

SEQ ID NO: 18 - protein, 8 aa, Homo sapiens
YDMVGIQG

SEQ ID NO: 19 - protein, 23 aa, Homo sapiens
HTANLCVLLYRSGVKVVTFCGHT

SEQ ID NO: 20 - protein, 9 aa, Homo sapiens
RSGVKVVTF

SEQ ID NO: 21 - protein, 121 aa, synthetic construct
QVQLQQPGAELVKPGASVKLSCKSSGYHFTSYWMHWVKQRPGQGLEWIGVIHPNSGSINYNEKFESKATLTVDKSSSTAYMQLSSLTSEDSAVYYCAGERDSTEVLPMDYWGQGTSVTVSS

SEQ ID NO: 22 - protein, 107 aa, synthetic construct
DVQITQSPSYLAASPGETITINCRASKSINKYLAWYQEKPGKTNKLLIYSGSTLQSGIPSRFSGSGSGTDFTLTISSLEPEDFAMYYCQQHNEYPLTFGAGTKLELK

SEQ ID NO: 23 - protein, 10 aa, synthetic construct
GYHFTSYWMH

SEQ ID NO: 24 - protein, 17 aa, synthetic construct
VIHPNSGSINYNEKFES

SEQ ID NO: 25 - protein, 12 aa, synthetic construct
ERDSTEVLPMDY

SEQ ID NO: 26 - DNA, 363 bp, synthetic construct
  source 1..363: mol_type = other DNA
caggtgcagctggtgcagtcaggggctgagctgaagaagcctggggcttcagtgaaggtttcctgcaagtcttctggctaccatttcaccagctactggatgcactgggtgaagcaggcccctggacaaggccttgagtggattggagtgattcatcctaatagtggtagtattaactacaatgagaagttcgagagcaaggccacaattactgtagacaaatccaccagcacagcctacatgcaactcagcagcctgacatctgaggactcggcggtctattattgtgcaggagagagagattctacggaggttctccctatggactactggggtcaaggaacctcagtcaccgtctcctca

SEQ ID NO: 27 - DNA, 363 bp, synthetic construct
  source 1..363: mol_type = other DNA
caggtgcagctggtgcagtcaggggctgagctgaagaagcctggggcttcagtgaaggtttcctgcaagtcttctggctaccatttcaccagctactggatgcactgggtgaagcaggcccctggacaaggccttgagtggattggagtgattcatcctaatagtggtagtattaactacaatgagaagttcgagagcagagccacaattactgtagacaaatccaccagcacagcctacatggagctcagcagcctgagatctgaggacacggcggtctattattgtgcaggagagagagattctacggaggttctccctatggactactggggtcaaggaaccacggtcaccgtctcctca

SEQ ID NO: 28 - DNA, 364 bp, synthetic construct
  source 1..364: mol_type = other DNA
caggtgcagctggtgcagtcaggggctgagctgaagaagcctggggcttcagtgaaggtttcctgcaagtcttctggctaccatttcaccagctactggatgcactgggtgaagcaggcccctggacaaggccttgagtggattggagtgattcatcctaatagtggtagtattaactacaatgagaagttcgagagcagagtcacaattactgtagacaaatccaccagcacagcctacatggagctcagcagcctgagatctgaggacacggcggtctattattgtgcaggagagagagattctacggaggttctccctatggactactggggtcaaggaaccacggtcaccgtctcctcag

SEQ ID NO: 29 - DNA, 363 bp, synthetic construct
  source 1..363: mol_type = other DNA
caggtgcagctggtgcagtcaggggctgagctgaagaagcctggggcttcagtgaaggtttcctgcaagtcttctggctaccatttcaccagctactggatgcactgggtgcgacaggcccctggacaaggccttgagtggattggagtgattcatcctaatagtggtagtattaactacaatgagaagttcgagagcagagtcacaattactgtagacaaatccaccagcacagcctacatggagctcagcagcctgagatctgaggacacggcggtctattattgtgcaggagagagagattctacggaggttctccctatggactactggggtcaaggaaccacggtcaccgtctcctca

SEQ ID NO: 30 - protein, 11 aa, synthetic construct
RASKSINKYLA

SEQ ID NO: 31 - protein, 7 aa, synthetic construct
SGSTLQS

SEQ ID NO: 32 - protein, 9 aa, synthetic construct
QQHNEYPLT

SEQ ID NO: 33 - DNA, 321 bp, synthetic construct
  source 1..321: mol_type = other DNA
gatgtccagatcacacagtctccatcttatcttgctgcatctctcggagaaagagctactattaattgcagggcaagtaagagcattaacaaatacttagcctggtatcaacagaaacctgggaaaactaataagctccttatctactctggctccactttgcaatctggaattccagcaaggttcagtggcagtggatctggtacagatttcactctcaccatcagtagcctggagcctgaagattttgcaatgtattactgtcaacaacataatgaatacccgctcacgttcggtcaggggaccaagctggagatcaaa

SEQ ID NO: 34 - DNA, 321 bp, synthetic construct
  source 1..321: mol_type = other DNA
gatgtccagatcacacagtctccatcttccctttctgcatctctcggagaaagagctactattaattgcagggcaagtaagagcattaacaaatacttagcctggtatcaacagaaacctgggaaagctaataagctccttatctactctggctccactttgcaatctggaattccagcaaggttcagtggcagtggatctggtacagatttcactctcaccatcagtagcctggagcctgaagattttgcaatgtattactgtcaacaacataatgaatacccgctcacgttcggtcaggggaccaagctggagatcaaa

SEQ ID NO: 35 - DNA, 321 bp, synthetic construct
  source 1..321: mol_type = other DNA
gatgtccagatcacacagtctccatcttccctttctgcatctctcggagaaagagctactattaattgcagggcaagtaagagcattaacaaatacttagcctggtatcaacagaaacctgggaaagctcctaagctccttatctactctggctccactttgcaatctggaattccagcaaggttcagtggcagtggatctggtacagatttcactctcaccatcagtagcctggagcctgaagattttgcaatgtattactgtcaacaacataatgaatacccgctcacgttcggtcaggggaccaagctggagatcaaa

SEQ ID NO: 36 - DNA, 321 bp, synthetic construct
  source 1..321: mol_type = other DNA
gatattcagctcacacagtctccatcttccctttctgcatctctcggagaaagagctactattaattgcagggcaagtaagagcattaacaaatacttagcctggtatcaacagaaacctgggaaagctcctaagctccttatctactctggctccactttgcaatctggaattccagcaaggttcagtggcagtggatctggtacagatttcactctcaccatcagtagcctggagcctgaagattttgcaatgtattactgtcaacaacataatgaatacccgctcacgttcggtcaggggaccaagctggagatcaaa

SEQ ID NO: 37 - protein, 327 aa, synthetic construct
ASTKGPSVFPLAPCSRSTSESTAALGCLVKDYFPEPVTVSWNSGALTSGVHTFPAVLQSSGLYSLSSVVTVPSSSLGTKTYTCNVDHKPSNTKVDKRVESKYGPPCPPCPAPEFEGGPSVFLFPPKPKDTLMISRTPEVTCVVVDVSQEDPEVQFNWYVDGVEVHNAKTKPREEQFNSTYRVVSVLTVLHQDWLNGKEYKCKVSNKGLPSSIEKTISKAKGQPREPQVYTLPPSQEEMTKNQVSLTCLVKGFYPSDIAVEWESNGQPENNYKTTPPVLDSDGSFFLYSRLTVDKSRWQEGNVFSCSVMHEALHNHYTQKSLSLSLGK

SEQ ID NO: 38 - protein, 98 aa, synthetic construct
ASTKGPSVFPLAPCSRSTSESTAALGCLVKDYFPEPVTVSWNSGALTSGVHTFPAVLQSSGLYSLSSVVTVPSSSLGTKTYTCNVDHKPSNTKVDKRV

SEQ ID NO: 39 - protein, 12 aa, synthetic construct
ESKYGPPCPPCP

SEQ ID NO: 40 - protein, 110 aa, synthetic construct
APEFEGGPSVFLFPPKPKDTLMISRTPEVTCVVVDVSQEDPEVQFNWYVDGVEVHNAKTKPREEQFNSTYRVVSVLTVLHQDWLNGKEYKCKVSNKGLPSSIEKTISKAK

SEQ ID NO: 41 - protein, 107 aa, synthetic construct
GQPREPQVYTLPPSQEEMTKNQVSLTCLVKGFYPSDIAVEWESNGQPENNYKTTPPVLDSDGSFFLYSRLTVDKSRWQEGNVFSCSVMHEALHNHYTQKSLSLSLGK

SEQ ID NO: 42 - DNA, 1805 bp, synthetic construct
  source 1..1805: mol_type = other DNA
gtaagctttctggggcaggccgggcctgactttggctgggggcagggagggggctaaggtgacgcaggtggcgccagccaggtgcacacccaatgcccatgagcccagacactggaccctgcatggaccatcgcggatagacaagaaccgaggggcctctgcgccctgggcccagctctgtcccacaccgcggtcacatggcaccacctctcttgcagcttccaccaagggcccatccgtcttccccctggcgccctgctccaggagcacctccgagagcacagccgccctgggctgcctggtcaaggactacttccccgaaccggtgacggtgtcgtggaactcaggcgccctgaccagcggcgtgcacaccttcccggctgtcctacagtcctcaggactctactccctcagcagcgtggtgaccgtgccctccagcagcttgggcacgaagacctacacctgcaatgtagatcacaagcccagcaacaccaaggtggacaagagagttggtgagaggccagcacagggagggagggtgtctgctggaagccaggctcagccctcctgcctggacgcaccccggctgtgcagccccagcccagggcagcaaggcaggccccatctgtctcctcacctggaggcctctgaccaccccactcatgctcagggagagggtcttctggatttttccaccaggctccgggcagccacaggctggatgcccctaccccaggccctgcgcatacaggggcaggtgctgcgctcagacctgccaagagccatatccgggaggaccctgcccctgacctaagcccaccccaaaggccaaactctccactccctcagctcagacaccttctctcctcccagatctgagtaactcccaatcttctctctgcagagtccaaatatggtcccccatgcccaccatgcccaggtaagccaacccaggcctcgccctccagctcaaggcgggacaggtgccctagagtagcctgcatccagggacaggccccagccgggtgctgacgcatccacctccatctcttcctcagcacctgagttcgaggggggaccatcagtcttcctgttccccccaaaacccaaggacactctcatgatctcccggacccctgaggtcacgtgcgtggtggtggacgtgagccaggaagaccccgaggtccagttcaactggtacgtggatggcgtggaggtgcataatgccaagacaaagccgcgggaggagcagttcaacagcacgtaccgtgtggtcagcgtcctcaccgtcctgcaccaggactggctgaacggcaaggagtacaagtgcaaggtctccaacaaaggcctcccgtcctccatcgagaaaaccatctccaaagccaaaggtgggacccacggggtgcgagggccacatggacagaggtcagctcggcccaccctctgccctgggagtgaccgctgtgccaacctctgtccctacagggcagccccgagagccacaggtgtacaccctgcccccatcccaggaggagatgaccaagaaccaggtcagcctgacctgcctggtcaaaggcttctaccccagcgacatcgccgtggagtgggagagcaatgggcagccggagaacaactacaagaccacgcctcccgtgctggactccgacggctccttcttcctctacagcaggctaaccgtggacaagagcaggtggcaggaggggaatgtcttctcatgctccgtgatgcatgaggctctgcacaaccactacacacagaagagcctctccctgtctctgggtaaa

SEQ ID NO: 43 - DNA, 294 bp, synthetic construct
  source 1..294: mol_type = other DNA
cttccaccaagggcccatccgtcttccccctggcgccctgctccaggagcacctccgagagcacagccgccctgggctgcctggtcaaggactacttccccgaaccggtgacggtgtcgtggaactcaggcgccctgaccagcggcgtgcacaccttcccggctgtcctacagtcctcaggactctactccctcagcagcgtggtgaccgtgccctccagcagcttgggcacgaagacctacacctgcaatgtagatcacaagcccagcaacaccaaggtggacaagagagttg

SEQ ID NO: 44 - DNA, 36 bp, synthetic construct
  source 1..36: mol_type = other DNA
agtccaaatatggtcccccatgcccaccatgcccag

SEQ ID NO: 45 - DNA, 330 bp, synthetic construct
  source 1..330: mol_type = other DNA
cacctgagttcgaggggggaccatcagtcttcctgttccccccaaaacccaaggacactctcatgatctcccggacccctgaggtcacgtgcgtggtggtggacgtgagccaggaagaccccgaggtccagttcaactggtacgtggatggcgtggaggtgcataatgccaagacaaagccgcgggaggagcagttcaacagcacgtaccgtgtggtcagcgtcctcaccgtcctgcaccaggactggctgaacggcaaggagtacaagtgcaaggtctccaacaaaggcctcccgtcctccatcgagaaaaccatctccaaagccaaag

SEQ ID NO: 46 - DNA, 320 bp, synthetic construct
  source 1..320: mol_type = other DNA
ggcagccccgagagccacaggtgtacaccctgcccccatcccaggaggagatgaccaagaaccaggtcagcctgacctgcctggtcaaaggcttctaccccagcgacatcgccgtggagtgggagagcaatgggcagccggagaacaactacaagaccacgcctcccgtgctggactccgacggctccttcttcctctacagcaggctaaccgtggacaagagcaggtggcaggaggggaatgtcttctcatgctccgtgatgcatgaggctctgcacaaccactacacacagaagagcctctccctgtctctgggtaaa